European Patent Application EP 4 296 282 A1, published December 27, 2023. Title: Single domain antibodies against CD47 and use thereof. Applicant: SNU R&DB Foundation Shaperon. The sequence listing filed with the application follows.

SEQUENCE LISTING (19 sequences)

SEQ ID NO: 1 - protein, 123 aa, Artificial Sequence
  CD47 Nb#01
QVQLVESGGGLVQPGGSLNLSCAVSGLTFFRKYAVGWARQVPGKGLERVSRIYSDRRIEYLDAVKGRFTISRDNAKNTVYLQMNSLKTEDTAVYYCATGLRVGLTGWDEYDYWGQGTQVTVSS

SEQ ID NO: 2 - protein, 125 aa, Artificial Sequence
  CD47 Nb#02
QVQLVESGGGLVQPGGSLRLSCTASGSTLNYYIISWFRQTPGKEREGVSCIGSSGAGTNYAASVKGRFTISRDDAQNTVYLFMNDLKPEDTAVYYCAARPFSFSPFCTFAGMKDWGKGTLVTVSS

SEQ ID NO: 3 - protein, 9 aa, Artificial Sequence
  CD47 Nb#01_CDR1
GLTFFRKYA

SEQ ID NO: 4 - protein, 7 aa, Artificial Sequence
  CD47 Nb#01_CDR2
IYSDRRI

SEQ ID NO: 5 - protein, 16 aa, Artificial Sequence
  CD47 Nb#01_CDR3
ATGLRVGLTGWDEYDY

SEQ ID NO: 6 - protein, 8 aa, Artificial Sequence
  CD47 Nb#02_CDR1
GSTLNYYI

SEQ ID NO: 7 - protein, 8 aa, Artificial Sequence
  CD47 Nb#02_CDR2
IGSSGAGT

SEQ ID NO: 8 - protein, 18 aa, Artificial Sequence
  CD47 Nb#02_CDR3
AARPFSFSPFCTFAGMKD

SEQ ID NO: 9 - protein, 360 aa, Artificial Sequence
  CD47 Nb#01-IgG1
QVQLVESGGGLVQPGGSLNLSCAVSGLTFFRKYAVGWARQVPGKGLERVSRIYSDRRIEYLDAVKGRFTISRDNAKNTVYLQMNSLKTEDTAVYYCATGLRVGLTGWDEYDYWGQGTQVTVSSGPGGPEPKSSDKTHTCPPCPAPELLGGPSVFLFPPKPKDTLMISRTPEVTCVVVDVSHEDPEVKFNWYVDGVEVHNAKTKPREEQYNSTYRVVSVLTVLHQDWLNGKEYKCKVSNKALPAPIEKTISKAKGQPREPQVYTLPPSRDELTKNQVSLTCLVKGFYPSDIAVEWESNGQPENNYKTTPPVLDSDGSFFLYSKLTVDKSRWQQGNVFSCSVMHEALHNHYTQKSLSLSPGK

SEQ ID NO: 10 - protein, 362 aa, Artificial Sequence
  CD47 Nb#02-IgG1
QVQLVESGGGLVQPGGSLRLSCTASGSTLNYYIISWFRQTPGKEREGVSCIGSSGAGTNYAASVKGRFTISRDDAQNTVYLFMNDLKPEDTAVYYCAARPFSFSPFCTFAGMKDWGKGTLVTVSSGPGGPEPKSSDKTHTCPPCPAPELLGGPSVFLFPPKPKDTLMISRTPEVTCVVVDVSHEDPEVKFNWYVDGVEVHNAKTKPREEQYNSTYRVVSVLTVLHQDWLNGKEYKCKVSNKALPAPIEKTISKAKGQPREPQVYTLPPSRDELTKNQVSLTCLVKGFYPSDIAVEWESNGQPENNYKTTPPVLDSDGSFFLYSKLTVDKSRWQQGNVFSCSVMHEALHNHYTQKSLSLSPGK

SEQ ID NO: 11 - protein, 25 aa, Artificial Sequence
  CD47 Nb#01_FR1
QVQLVESGGGLVQPGGSLNLSCAVS

SEQ ID NO: 12 - protein, 17 aa, Artificial Sequence
  CD47 Nb#01_FR2
VGWARQVPGKGLERVSR

SEQ ID NO: 13 - protein, 38 aa, Artificial Sequence
  CD47 Nb#01_FR3
EYLDAVKGRFTISRDNAKNTVYLQMNSLKTEDTAVYYC

SEQ ID NO: 14 - protein, 11 aa, Artificial Sequence
  CD47 Nb#01_FR4
WGQGTQVTVSS

SEQ ID NO: 15 - protein, 25 aa, Artificial Sequence
  CD47 Nb#02_FR1
QVQLVESGGGLVQPGGSLRLSCTAS

SEQ ID NO: 16 - protein, 17 aa, Artificial Sequence
  CD47 Nb#02_FR2
ISWFRQTPGKEREGVSC

SEQ ID NO: 17 - protein, 38 aa, Artificial Sequence
  CD47 Nb#02_FR3
NYAASVKGRFTISRDDAQNTVYLFMNDLKPEDTAVYYC

SEQ ID NO: 18 - protein, 11 aa, Artificial Sequence
  CD47 Nb#02_FR4
WGKGTLVTVSS

SEQ ID NO: 19 - protein, 357 aa, Artificial Sequence
  CD47 Nb-IgG4
QVQLVESGGGLVQPGGSLNLSCAVSGLTFFRKYAVGWARQVPGKGLERVSRIYSDRRIEYLDAVKGRFTISRDNAKNTVYLQMNSLKTEDTAVYYCATGLRVGLTGWDEYDYWGQGTQVTVSSGPGGPESKYGPPCPPCPAPEFLGGPSVFLFPPKPKDTLMISRTPEVTCVVVDVSQEDPEVQFNWYVDGVEVHNAKTKPREEQFNSTYRVVSVLTVLHQDWLNGKEYKCKVSNKGLPSSIEKTISKAKGQPREPQVYTLPPSQEEMTKNQVSLTCLVKGFYPSDIAVEWESNGQPENNYKTTPPVLDSDGSFFLYSRLTVDKSRWQEGNVFSCSVMHEALHNHYTQKSLSLSPGK